European Patent Specification EP 3 519 830 B1, published July 19, 2023. Title: Kinase reporter. Applicant: Universität Innsbruck. The sequence listing filed with the application follows.

SEQUENCE LISTING (34 sequences)

SEQ ID NO: 1 - protein, 608 aa, Homo sapiens
MEPPRGPPANGAEPSRAVGTVKVYLPNKQRTVVTVRDGMSVYDSLDKALKVRGLNQDCCVVYRLIKGRKTVTAWDTAIAPLDGEELIVEVLEDVPLTMHNFVRKTFFSLAFCDFCLKFLFHGFRCQTCGYKFHQHCSSKVPTVCVDMSTNRQQFYHSVQDLSGGSRQHEAPSNRPLNELLTPQGPSPRTQHCDPEHFPFPAPANAPLQRIRSTSTPNVHMVSTTAPMDSNLIQLTGQSFSTDAAGSRGGSDGTPRGSPSPASVSSGRKSPHSKSPAEQRERKSLADDKKKVKNLGYRDSGYYWEVPPSEVQLLKRIGTGSFGTVFRGRWHGDVAVKVLKVSQPTAEQAQAFKNEMQVLRKTRHVNILLFMGFMTRPGFAIITQWCEGSSLYHHLHVADTRFDMVQLIDVARQTAQGMDYLHAKNIIHRDLKSNNIFLHEGLTVKIGDFGLATVKTRWSGAQPLEQPSGSVLWMAAEVIRMQDPNPYSFQSDVYAYGVVLYELMTGSLPYSHIGCRDQIIFMVGRGYLSPDLSKISSNCPKAMRRLLSDCLKFQREERPLFPQILATIELLQRSLPKIERSASEPSLHRTQADELPACLLSAARLVPID

SEQ ID NO: 2 - protein, 768 aa, Homo sapiens
MAALSGGGGGGAEPGQALFNGDMEPEAGAGAGAAASSAADPAIPEEVWNIKQMIKLTQEHIEALLDKFGGEHNPPSIYLEAYEEYTSKLDALQQREQQLLESLGNGTDFSVSSSASMDTVTSSSSSSLSVLPSSLSVFQNPTDVARSNPKSPQKPIVRVFLPNKQRTVVPARCGVTVRDSLKKALMMRGLIPECCAVYRIQDGEKKPIGWDTDISWLTGEELHVEVLENVPLTTHNFVRKTFFTLAFCDFCRKLLFQGFRCQTCGYKFHQRCSTEVPLMCVNYDQLDLLFVSKFFEHHPIPQEEASLAETALTSGSSPSAPASDSIGPQILTSPSPSKSIPIPQPFRPADEDHRNQFGQRDRSSSAPNVHINTIEPVNIDDLIRDQGFRGDGGSTTGLSATPPASLPGSLTNVKALQKSPGPQRERKSSSSSEDRNRMKTLGRRDSSDDWEIPDGQITVGQRIGSGSFGTVYKGKWHGDVAVKMLNVTAPTPQQLQAFKNEVGVLRKTRHVNILLFMGYSTKPQLAIVTQWCEGSSLYHHLHIIETKFEMIKLIDIARQTAQGMDYLHAKSIIHRDLKSNNIFLHEDLTVKIGDFGLATVKSRWSGSHQFEQLSGSILWMAPEVIRMQDKNPYSFQSDVYAFGIVLYELMTGQLPYSNINNRDQIIFMVGRGYLSPDLSKVRSNCPKAMKRLMAECLKKKRDERPLFPQILASIELLARSLPKIHRSASEPSLNRAGFQTEDFSLYACASPKTPIQAGGYGAFPVHID

SEQ ID NO: 3 - protein, 650 aa, Homo sapiens
MEHIQGAWKTISNGFGFKDAVFDGSSCISPTIVQQFGYQRRASDDGKLTDPSKTSNTIRVFLPNKQRTVVNVRNGMSLHDCLMKALKVRGLQPECCAVFRLLHEHKGKKARLDWNTDAASLIGEELQVDFLDHVPLTTHNFARKTFLKLAFCDICQKFLLNGFRCQTCGYKFHEHCSTKVPTMCVDWSNIRQLLLFPNSTIGDSGVPALPSLTMRRMRESVSRMPVSSQHRYSTPHAFTFNTSSPSSEGSLSQRQRSTSTPNVHMVSTTLPVDSRMIEDAIRSHSESASPSALSSSPNNLSPTGWSQPKTPVPAQRERAPVSGTQEKNKIRPRGQRDSSYYWEIEASEVMLSTRIGSGSFGTVYKGKWHGDVAVKILKVVDPTPEQFQAFRNEVAVLRKTRHVNILLFMGYMTKDNLAIVTQWCEGSSLYKHLHVQETKFQMFQLIDIARQTAQGMDYLHAKNIIHRDMKSNNIFLHEGLTVKIGDFGLATVKSRWSGSQQVEQPTGSVLWMAPEVIRMQDNNPFSFQSDVYSYGIVLYELMTGELPYSHINNRDQIIFMVGRGYASPDLSKLYKNCPKAMKRLVADCVKKVKEERPLFPQILSSIELLQHSLPKINRSASEPSLHRAAHTEDINACTLTTSPRLPVFID

SEQ ID NO: 4 - protein, 608 aa, Homo sapiens
MEPPRGPPANGAEPSRAVGTVKVYLPNKQRTVVTVRDGMSVYDSLDKALKVRGLNQDCCVVYRLIKGRKTVTAWDTAIAPLDGEELIVEVLEDVPLTMHNFVRKTFFSLAFCDFCLKFLFHGFRCQTCGYKFHQHCSSKVPTVCVDMSTNRQQFYHSVQDLSGGSRQHEAPSNRPLNELLTPQGPSPRTQHCDPEHFPFPAPANAPLQRIRSTCTPNVHMVSTTAPMDSNLIQLTGQSFSTDAAGSRGGSDGTPRGSPSPASVSSGRKSPHSKSPAEQRERKSLADDKKKVKNLGYRDSGYYWEVPPSEVQLLKRIGTGSFGTVFRGRWHGDVAVKVLKVSQPTAEQAQAFKNEMQVLRKTRHVNILLFMGFMTRPGFAIITQWCEGSSLYHHLHVADTRFDMVQLIDVARQTAQGMDYLHAKNIIHRDLKSNNIFLHEGLTVKIGDFGLATVKTRWSGAQPLEQPSGSVLWMAAEVIRMQDPNPYSFQSDVYAYGVVLYELMTGSLPYSHIGCRDQIIFMVGRGYLSPDLSKISSNCPKAMRRLLSDCLKFQREERPLFPQILATIELLQRSLPKIERSASEPSLHRTQADELPACLLSAARLVPID

SEQ ID NO: 5 - protein, 768 aa, Homo sapiens
MAALSGGGGGGAEPGQALFNGDMEPEAGAGAGAAASSAADPAIPEEVWNIKQMIKLTQEHIEALLDKFGGEHNPPSIYLEAYEEYTSKLDALQQREQQLLESLGNGTDFSVSSSASMDTVTSSSSSSLSVLPSSLSVFQNPTDVARSNPKSPQKPIVRVFLPNKQRTVVPARCGVTVRDSLKKALMMRGLIPECCAVYRIQDGEKKPIGWDTDISWLTGEELHVEVLENVPLTTHNFVRKTFFTLAFCDFCRKLLFQGFRCQTCGYKFHQRCSTEVPLMCVNYDQLDLLFVSKFFEHHPIPQEEASLAETALTSGSSPSAPASDSIGPQILTSPSPSKSIPIPQPFRPADEDHRNQFGQRDRSSSAPNVHINTIEPVNIDDLIRDQGFRGDGGSTTGLSATPPASLPGSLTNVKALQKSPGPQRERKSSSSSEDRNRMKTLGRRDSSDDWEIPDGQITVGQRIGSGSFGTVYKGKWHGDVAVKMLNVTAPTPQQLQAFKNEVGVLRKTRHVNILLFMGYSTKPQLAIVTQWCEGSSLYHHLHIIETKFEMIKLIDIARQTAQGMDYLHAKSIIHRDLKSNNIFLHEDLTVKIGDFGLATEKSRWSGSHQFEQLSGSILWMAPEVIRMQDKNPYSFQSDVYAFGIVLYELMTGQLPYSNINNRDQIIFMVGRGYLSPDLSKVRSNCPKAMKRLMAECLKKKRDERPLFPQILASIELLARSLPKIHRSASEPSLNRAGFQTEDFSLYACASPKTPIQAGGYGAFPVHID

SEQ ID NO: 6 - protein, 768 aa, Homo sapiens
MAALSGGGGGGAEPGQALFNGDMEPEAGAGAGAAASSAADPAIPEEVWNIKQMIKLTQEHIEALLDKFGGEHNPPSIYLEAYEEYTSKLDALQQREQQLLESLGNGTDFSVSSSASMDTVTSSSSSSLSVLPSSLSVFQNPTDVARSNPKSPQKPIVRVFLPNKQRTVVPARCGVTVRDSLKKALMMRGLIPECCAVYRIQDGEKKPIGWDTDISWLTGEELHVEVLENVPLTTHNFVRKTFFTLAFCDFCRKLLFQGFRCQTCGYKFHQRCSTEVPLMCVNYDQLDLLFVSKFFEHHPIPQEEASLAETALTSGSSPSAPASDSIGPQILTSPSPSKSIPIPQPFRPADEDHRNQFGQRDRSSSAPNVHINTIEPVNIDDLIRDQGFRGDGGSTTGLSATPPASLPGSLTNVKALQKSPGPQRERKSSSSSEDRNRMKTLGRRDSSDDWEIPDGQITVGQRIGSGSFGTVYKGKWHGDVAVKMLNVTAPTPQQLQAFKNEVGVLRKTRHVNILLFMGYSTKPQLAIVTQWCEGSSLYHHLHIIETKFEMIKLIDIARQTAQGMDYLHAKSIIHRDLKSNNIFLHEDLTVKIGDFGLATKKSRWSGSHQFEQLSGSILWMAPEVIRMQDKNPYSFQSDVYAFGIVLYELMTGQLPYSNINNRDQIIFMVGRGYLSPDLSKVRSNCPKAMKRLMAECLKKKRDERPLFPQILASIELLARSLPKIHRSASEPSLNRAGFQTEDFSLYACASPKTPIQAGGYGAFPVHID

SEQ ID NO: 7 - protein, 768 aa, Homo sapiens
MAALSGGGGGGAEPGQALFNGDMEPEAGAGAGAAASSAADPAIPEEVWNIKQMIKLTQEHIEALLDKFGGEHNPPSIYLEAYEEYTSKLDALQQREQQLLESLGNGTDFSVSSSASMDTVTSSSSSSLSVLPSSLSVFQNPTDVARSNPKSPQKPIVRVFLPNKQRTVVPARCGVTVRDSLKKALMMRGLIPECCAVYRIQDGEKKPIGWDTDISWLTGEELHVEVLENVPLTTHNFVRKTFFTLAFCDFCRKLLFQGFRCQTCGYKFHQRCSTEVPLMCVNYDQLDLLFVSKFFEHHPIPQEEASLAETALTSGSSPSAPASDSIGPQILTSPSPSKSIPIPQPFRPADEDHRNQFGQRDRSSSAPNVHINTIEPVNIDDLIRDQGFRGDGGSTTGLSATPPASLPGSLTNVKALQKSPGPQRERKSSSSSEDRNRMKTLGRRDSSDDWEIPDGQITVGQRIGSGSFGTVYKGKWHGDVAVKMLNVTAPTPQQLQAFKNEVGVLRKTRHVNILLFMGYSTKPQLAIVTQWCEGSSLYHHLHIIETKFEMIKLIDIARQTAQGMDYLHAKSIIHRDLKSNNIFLHEDLTVKIGDFGLATRKSRWSGSHQFEQLSGSILWMAPEVIRMQDKNPYSFQSDVYAFGIVLYELMTGQLPYSNINNRDQIIFMVGRGYLSPDLSKVRSNCPKAMKRLMAECLKKKRDERPLFPQILASIELLARSLPKIHRSASEPSLNRAGFQTEDFSLYACASPKTPIQAGGYGAFPVHID

SEQ ID NO: 8 - protein, 768 aa, Homo sapiens
MAALSGGGGGGAEPGQALFNGDMEPEAGAGAGAAASSAADPAIPEEVWNIKQMIKLTQEHIEALLDKFGGEHNPPSIYLEAYEEYTSKLDALQQREQQLLESLGNGTDFSVSSSASMDTVTSSSSSSLSVLPSSLSVFQNPTDVARSNPKSPQKPIVRVFLPNKQRTVVPARCGVTVRDSLKKALMMRGLIPECCAVYRIQDGEKKPIGWDTDISWLTGEELHVEVLENVPLTTHNFVRKTFFTLAFCDFCRKLLFQGFRCQTCGYKFHQRCSTEVPLMCVNYDQLDLLFVSKFFEHHPIPQEEASLAETALTSGSSPSAPASDSIGPQILTSPSPSKSIPIPQPFRPADEDHRNQFGQRDRSSSAPNVHINTIEPVNIDDLIRDQGFRGDGGSTTGLSATPPASLPGSLTNVKALQKSPGPQRERKSSSSSEDRNRMKTLGRRDSSDDWEIPDGQITVGQRIGSGSFGTVYKGKWHGDVAVKMLNVTAPTPQQLQAFKNEVGVLRKTRHVNILLFMGYSTKPQLAIVTQWCEGSSLYHHLHIIETKFEMIKLIDIARQTAQGMDYLHAKSIIHRDLKSNNIFLHEDLTVKIGGFGLATVKSRWSGSHQFEQLSGSILWMAPEVIRMQDKNPYSFQSDVYAFGIVLYELMTGQLPYSNINNRDQIIFMVGRGYLSPDLSKVRSNCPKAMKRLMAECLKKKRDERPLFPQILASIELLARSLPKIHRSASEPSLNRAGFQTEDFSLYACASPKTPIQAGGYGAFPVHID

SEQ ID NO: 9 - protein, 768 aa, Homo sapiens
MAALSGGGGGGAEPGQALFNGDMEPEAGAGAGAAASSAADPAIPEEVWNIKQMIKLTQEHIEALLDKFGGEHNPPSIYLEAYEEYTSKLDALQQREQQLLESLGNGTDFSVSSSASMDTVTSSSSSSLSVLPSSLSVFQNPTDVARSNPKSPQKPIVRVFLPNKQRTVVPARCGVTVRDSLKKALMMRGLIPECCAVYRIQDGEKKPIGWDTDISWLTGEELHVEVLENVPLTTHNFVRKTFFTLAFCDFCRKLLFQGFRCQTCGYKFHQRCSTEVPLMCVNYDQLDLLFVSKFFEHHPIPQEEASLAETALTSGSSPSAPASDSIGPQILTSPSPSKSIPIPQPFRPADEDHRNQFGQRDRSSSAPNVHINTIEPVNIDDLIRDQGFRGDGGSTTGLSATPPASLPGSLTNVKALQKSPGPQRERKSSSSSEDRNRMKTLGRRDSSDDWEIPDGQITVGQRIGSGSFATVYKGKWHGDVAVKMLNVTAPTPQQLQAFKNEVGVLRKTRHVNILLFMGYSTKPQLAIVTQWCEGSSLYHHLHIIETKFEMIKLIDIARQTAQGMDYLHAKSIIHRDLKSNNIFLHEDLTVKIGDFGLATVKSRWSGSHQFEQLSGSILWMAPEVIRMQDKNPYSFQSDVYAFGIVLYELMTGQLPYSNINNRDQIIFMVGRGYLSPDLSKVRSNCPKAMKRLMAECLKKKRDERPLFPQILASIELLARSLPKIHRSASEPSLNRAGFQTEDFSLYACASPKTPIQAGGYGAFPVHID

SEQ ID NO: 10 - protein, 768 aa, Homo sapiens
MAALSGGGGGGAEPGQALFNGDMEPEAGAGAGAAASSAADPAIPEEVWNIKQMIKLTQEHIEALLDKFGGEHNPPSIYLEAYEEYTSKLDALQQREQQLLESLGNGTDFSVSSSASMDTVTSSSSSSLSVLPSSLSVFQNPTDVARSNPKSPQKPIVRVFLPNKQRTVVPARCGVTVRDSLKKALMMRGLIPECCAVYRIQDGEKKPIGWDTDISWLTGEELHVEVLENVPLTTHNFVRKTFFTLAFCDFCRKLLFQGFRCQTCGYKFHQRCSTEVPLMCVNYDQLDLLFVSKFFEHHPIPQEEASLAETALTSGSSPSAPASDSIGPQILTSPSPSKSIPIPQPFRPADEDHRNQFGQRDRSSSAPNVHINTIEPVNIDDLIRDQGFRGDGGSTTGLSATPPASLPGSLTNVKALQKSPGPQRERKSSSSSEDRNRMKTLGRRDSSDDWEIPDGQITVGQRIGSGSFGTVYKGKWHGDVAVKMLNVTAPTPQQLQAFKNEVGVLRKTRHVNILLFMGYSTKPQLAIVTQWCEGSSLYHHLHIIETKFEMIKLIDIARQTAQGMDYLHAKSIIHRDLKSNNIFLHEDLTVKIGDFGLATVESRWSGSHQFEQLSGSILWMAPEVIRMQDKNPYSFQSDVYAFGIVLYELMTGQLPYSNINNRDQIIFMVGRGYLSPDLSKVRSNCPKAMKRLMAECLKKKRDERPLFPQILASIELLARSLPKIHRSASEPSLNRAGFQTEDFSLYACASPKTPIQAGGYGAFPVHID

SEQ ID NO: 11 - protein, 650 aa, Homo sapiens
MEHIQGAWKTISNGFGFKDAVFDGSSCISPTIVQQFGYQRRASDDGKLTDPSKTSNTIRVFLPNKQRTVVNVRNGMSLHDCLMKALKVRGLQPECCAVFRLLHEHKGKKARLDWNTDAASLIGEELQVDFLDHVPLTTHNFARKTFLKLAFCDICQKFLLNGFRCQTCGYKFHEHCSTKVPTMCVDWSNIRQLLLFPNSTIGDSGVPALPSLTMRRMRESVSRMPVSSQHRYSTPHAFTFNTSSPSSEGSLSQRQRLTSTPNVHMVSTTLPVDSRMIEDAIRSHSESASPSALSSSPNNLSPTGWSQPKTPVPAQRERAPVSGTQEKNKIRPRGQRDSSYYWEIEASEVMLSTRIGSGSFGTVYKGKWHGDVAVKILKVVDPTPEQFQAFRNEVAVLRKTRHVNILLFMGYMTKDNLAIVTQWCEGSSLYKHLHVQETKFQMFQLIDIARQTAQGMDYLHAKNIIHRDMKSNNIFLHEGLTVKIGDFGLATVKSRWSGSQQVEQPTGSVLWMAPEVIRMQDNNPFSFQSDVYSYGIVLYELMTGELPYSHINNRDQIIFMVGRGYASPDLSKLYKNCPKAMKRLVADCVKKVKEERPLFPQILSSIELLQHSLPKINRSASEPSLHRAAHTEDINACTLTTSPRLPVFID

SEQ ID NO: 12 - protein, 650 aa, Homo sapiens
MEHIQGAWKTISNGFGFKDAVFDGSSCISPTIVQQFGYQRRASDDGKLTDPSKTSNTIRVFLPNKQRTVVNVRNGMSLHDCLMKALKVRGLQPECCAVFRLLHEHKGKKARLDWNTDAASLIGEELQVDFLDHVPLTTHNFARKTFLKLAFCDICQKFLLNGFRCQTCGYKFHEHCSTKVPTMCVDWSNIRQLLLFPNSTIGDSGVPALPSLTMRRMRESVSRMPVSSQHRYSTPHAFTFNTSSPSSEGSLSQRQRSTATPNVHMVSTTLPVDSRMIEDAIRSHSESASPSALSSSPNNLSPTGWSQPKTPVPAQRERAPVSGTQEKNKIRPRGQRDSSYYWEIEASEVMLSTRIGSGSFGTVYKGKWHGDVAVKILKVVDPTPEQFQAFRNEVAVLRKTRHVNILLFMGYMTKDNLAIVTQWCEGSSLYKHLHVQETKFQMFQLIDIARQTAQGMDYLHAKNIIHRDMKSNNIFLHEGLTVKIGDFGLATVKSRWSGSQQVEQPTGSVLWMAPEVIRMQDNNPFSFQSDVYSYGIVLYELMTGELPYSHINNRDQIIFMVGRGYASPDLSKLYKNCPKAMKRLVADCVKKVKEERPLFPQILSSIELLQHSLPKINRSASEPSLHRAAHTEDINACTLTTSPRLPVFID

SEQ ID NO: 13 - protein, 393 aa, Homo sapiens [sequence omitted]

SEQ ID NO: 14 - protein, 400 aa, Homo sapiens [sequence omitted]

SEQ ID NO: 15 - protein, 393 aa, Homo sapiens
MPKKKPTPIQLNPAPDGSAVNGTSSAETNLEALQKKLEELELDEQQRKRLEAFLTQKQKVGELKDDDFEKISELGAGNGGVVFKVSHKPSGLVMARKLIHLEIKPAIRNQIIRELQVLHECNSPYIVGFYGAFYSDGEISICMEHMDGGSLDQVLKKAGRIPEQILGKVSIAVIKGLTYLREKHKIMHRDVKPSNILVNSRGEIKLCDFGVSGQLIDAMANSFVGTRSYMSPERLQGTHYSVQSDIWSMGLSLVEMAVGRYPIPPPDAKELELMFGCQVEGDAAETPPRPRTPGRPLSSYGMDSRPPMAIFELLDYIVNEPPPKLPSGVFSLEFQDFVNKCLIKNPAERADLKQLMVHAFIKRSDAEEVDFAGWLCSTIGLNQPSTPTHAAGV

SEQ ID NO: 16 - protein, 393 aa, Homo sapiens
MPKKKPTPIQLNPAPDGSAVNGTSSAETNLEALQKKLEELELDEQQRKRLEAFLTQKQKVGELKDDDFEKISELGAGNGGVVFKVSHKPSGLVMARKLIHLEIKPAIRNQIIRELQVLHECNSPYIVGFYGAFYSDGEISICMEHMDGGSLDQVLKKAGRIPEQILGKVSIAVIKGLTYLREKHKIMHRDVKPSNILVNSRGEIKLCDFGVSGQLIDEMANEFVGTRSYMSPERLQGTHYSVQSDIWSMGLSLVEMAVGRYPIPPPDAKELELMFGCQVEGDAAETPPRPRTPGRPLSSYGMDSRPPMAIFELLDYIVNEPPPKLPSGVFSLEFQDFVNKCLIKNPAERADLKQLMVHAFIKRSDAEEVDFAGWLCSTIGLNQPSTPTHAAGV

SEQ ID NO: 17 - protein, 109 aa, Artificial sequence
  Luciferase fragement derived from Renilla luciferase protein sequence
ASKVYDPEQRKRMITGPQWWARCKQMNVLDSFINYYDSEKHAENAVIFLHGNAASSYLWRHVVPHIEPVARCIIPDLIGMGKSGKSGNGSYRLLDHYKYLTAWFELLNL

SEQ ID NO: 18 - protein, 201 aa, Artificial sequence
  Luciferase fragement derived from Renilla luciferase protein sequence
PKKIIFVGHDWGACLAFHYSYEHQDKIKAIVHAESVVDVIESWDEWPDIEEDIALIKSEEGEKMVLENNFFVETMLPSKIMRKLEPEEFAAYLEPFKEKGEVRRPTLSWPREIPLVKGGKPDVVQIVRNYNAYLRASDDLPKMFIESDPGFFSNAIVEGAKKFPNTEFVKVKGLHFSQEDAPDEMGKYIKSFVERVLKNEQ

SEQ ID NO: 19 - protein, 93 aa, Artificial sequence
  Luciferase fragement derived from Gaussia luciferase protein sequence
MKPTENNEDFNIVAVASNFATTDLDADRGKLPGKKLPLEVLKEMEANARKAGCTRGCLICLSHIKCTPKMKKFIPGRCHTYEGDKESAQGGIG

SEQ ID NO: 20 - protein, 76 aa, Artificial Sequence
  Luciferase fragement derived from Gaussia luciferase protein sequence
EAIVDIPEIPGFKDLEPMEQFIAQVDLCVDCTTGCLKGLANVQCSDLLKKWLPQRCATFASKIQGQVDKIKGAGGD

SEQ ID NO: 21 - protein, 10 aa, Artificial Sequence
  Potential linker for fused protein construct
GGGGSGGGGS

SEQ ID NO: 22 - protein, 1104 aa, Artificial sequence
  BRAF(wt) reporter comprising an N-terminal Renilla luciferase fragment, a linker, a BRAF(wt) sequence, a linker, and a C-terminal Renilla luciferase fragment
MASKVYDPEQRKRMITGPQWWARCKQMNVLDSFINYYDSEKHAENAVIFLHGNAASSYLWRHVVPHIEPVARCIIPDLIGMGKSGKSGNGSYRLLDHYKYLTAWFELLNLIDGGGGSGGGGSSGAALSGGGGGGAEPGQALFNGDMEPEAGAGAGAAASSAADPAIPEEVWNIKQMIKLTQEHIEALLDKFGGEHNPPSIYLEAYEEYTSKLDALQQREQQLLESLGNGTDFSVSSSASMDTVTSSSSSSLSVLPSSLSVFQNPTDVARSNPKSPQKPIVRVFLPNKQRTVVPARCGVTVRDSLKKALMMRGLIPECCAVYRIQDGEKKPIGWDTDISWLTGEELHVEVLENVPLTTHNFVRKTFFTLAFCDFCRKLLFQGFRCQTCGYKFHQRCSTEVPLMCVNYDQLDLLFVSKFFEHHPIPQEEASLAETALTSGSSPSAPASDSIGPQILTSPSPSKSIPIPQPFRPADEDHRNQFGQRDRSSSAPNVHINTIEPVNIDDLIRDQGFRGDGGSTTGLSATPPASLPGSLTNVKALQKSPGPQRERKSSSSSEDRNRMKTLGRRDSSDDWEIPDGQITVGQRIGSGSFGTVYKGKWHGDVAVKMLNVTAPTPQQLQAFKNEVGVLRKTRHVNILLFMGYSTKPQLAIVTQWCEGSSLYHHLHIIETKFEMIKLIDIARQTAQGMDYLHAKSIIHRDLKSNNIFLHEDLTVKIGDFGLATVKSRWSGSHQFEQLSGSILWMAPEVIRMQDKNPYSFQSDVYAFGIVLYELMTGQLPYSNINNRDQIIFMVGRGYLSPDLSKVRSNCPKAMKRLMAECLKKKRDERPLFPQILASIELLARSLPKIHRSASEPSLNRAGFQTEDFSLYACASPKTPIQAGGYGAFPVHSRGGGGSGGGGSSGPKKIIFVGHDWGACLAFHYSYEHQDKIKAIVHAESVVDVIESWDEWPDIEEDIALIKSEEGEKMVLENNFFVETMLPSKIMRKLEPEEFAAYLEPFKEKGEVRRPTLSWPREIPLVKGGKPDVVQIVRNYNAYLRASDDLPKMFIESDPGFFSNAIVEGAKKFPNTEFVKVKGLHFSQEDAPDEMGKYIKSFVERVLKNEQ

SEQ ID NO: 23 - protein, 731 aa, Artificial sequence
  MEK1(wt) reporter comprising an N-terminal Renilla luciferase fragment, a linker, a MEK1(wt) sequence, a linker, and a C-terminal Renilla luciferase fragment
MASKVYDPEQRKRMITGPQWWARCKQMNVLDSFINYYDSEKHAENAVIFLHGNAASSYLWRHVVPHIEPVARCIIPDLIGMGKSGKSGNGSYRLLDHYKYLTAWFELLNLIDGGGGSGGGGSSGPKKKPTPIQLNPAPDGSAVNGTSSAETNLEALQKKLEELELDEQQRKRLEAFLTQKQKVGELKDDDFEKISELGAGNGGVVFKVSHKPSGLVMARKLIHLEIKPAIRNQIIRELQVLHECNSPYIVGFYGAFYSDGEISICMEHMDGGSLDQVLKKAGRIPEQILGKVSIAVIKGLTYLREKHKIMHRDVKPSNILVNSRGEIKLCDFGVSGQLIDSMANSFVGTRSYMSPERLQGTHYSVQSDIWSMGLSLVEMAVGRYPIPPPDAKELELMFGCQVEGDAAETPPRPRTPGRPLSSYGMDSRPPMAIFELLDYIVNEPPPKLPSAVFSLEFQDFVNKCLIKNPAERADLKQLMVHAFIKRSDAEEVDFAGWLCSTIGLNQPSTPTHAAGVSRGGGGSGGGGSSGPKKIIFVGHDWGACLAFHYSYEHQDKIKAIVHAESVVDVIESWDEWPDIEEDIALIKSEEGEKMVLENNFFVETMLPSKIMRKLEPEEFAAYLEPFKEKGEVRRPTLSWPREIPLVKGGKPDVVQIVRNYNAYLRASDDLPKMFIESDPGFFSNAIVEGAKKFPNTEFVKVKGLHFSQEDAPDEMGKYIKSFVERVLKNEQ

SEQ ID NO: 24 - protein, 962 aa, Artificial Sequence
  BRAF(wt) reporter comprising an N-terminal Gaussia luciferase fragment, a linker, a BRAF(wt) sequence, a linker, and a C-terminal Gaussia luciferase fragment
MKPTENNEDFNIVAVASNFATTDLDADRGKLPGKKLPLEVLKEMEANARKAGCTRGCLICLSHIKCTPKMKKFIPGRCHTYEGDKESAQGGIGIDGGGGSGGGGSSGAALSGGGGGGAEPGQALFNGDMEPEAGAGAGAAASSAADPAIPEEVWNIKQMIKLTQEHIEALLDKFGGEHNPPSIYLEAYEEYTSKLDALQQREQQLLESLGNGTDFSVSSSASMDTVTSSSSSSLSVLPSSLSVFQNPTDVARSNPKSPQKPIVRVFLPNKQRTVVPARCGVTVRDSLKKALMMRGLIPECCAVYRIQDGEKKPIGWDTDISWLTGEELHVEVLENVPLTTHNFVRKTFFTLAFCDFCRKLLFQGFRCQTCGYKFHQRCSTEVPLMCVNYDQLDLLFVSKFFEHHPIPQEEASLAETALTSGSSPSAPASDSIGPQILTSPSPSKSIPIPQPFRPADEDHRNQFGQRDRSSSAPNVHINTIEPVNIDDLIRDQGFRGDGGSTTGLSATPPASLPGSLTNVKALQKSPGPQRERKSSSSSEDRNRMKTLGRRDSSDDWEIPDGQITVGQRIGSGSFGTVYKGKWHGDVAVKMLNVTAPTPQQLQAFKNEVGVLRKTRHVNILLFMGYSTKPQLAIVTQWCEGSSLYHHLHIIETKFEMIKLIDIARQTAQGMDYLHAKSIIHRDLKSNNIFLHEDLTVKIGDFGLATVKSRWSGSHQFEQLSGSILWMAPEVIRMQDKNPYSFQSDVYAFGIVLYELMTGQLPYSNINNRDQIIFMVGRGYLSPDLSKVRSNCPKAMKRLMAECLKKKRDERPLFPQILASIELLARSLPKIHRSASEPSLNRAGFQTEDFSLYACASPKTPIQAGGYGAFPVHSRGGGGSGGGGSSGEAIVDIPEIPGFKDLEPMEQFIAQVDLCVDCTTGCLKGLANVQCSDLLKKWLPQRCATFASKIQGQVDKIKGAGGD

SEQ ID NO: 25 - protein, 194 aa, Homo sapiens
MEEKLKKTKIIFVVGGPGSGKGTQCEKIVQKYGYTHLSTGDLLRSEVSSGSARGKKLSEIMEKGQLVPLETVLDMLRDAMVAKVNTSKGFLIDGYPREVQQGEEFERRIGQPTLLLYVDAGPETMTQRLLKRGETSGRVDDNEETIKKRLETYYKATEPVIAFYEKRGIVRKVNAEGSVDSVFSQVCTHLDALK

SEQ ID NO: 26 - protein, 303 aa, Homo sapiens
MATSRYEPVAEIGVGAYGTVYKARDPHSGHFVALKSVRVPNGGGGGGGLPISTVREVALLRRLEAFEHPNVVRLMDVCATSRTDREIKVTLVFEHVDQDLRTYLDKAPPPGLPAETIKDLMRQFLRGLDFLHANCIVHRDLKPENILVTSGGTVKLADFGLARIYSYQMALTPVVVTLWYRAPEVLLQSTYATPVDMWSVGCIFAEMFRRKPLFCGNSEADQLGKIFDLIGLPPEDDWPRDVSLPRGAFPPRGPRPVQSVVPEMEESGAQLLLEMLTFNPHKRISAFRALQHSYLHKDEGNPE

SEQ ID NO: 27 - protein, 420 aa, Homo sapiens
MSGRPRTTSFAESCKPVQQPSAFGSMKVSRDKDGSKVTTVVATPGQGPDRPQEVSYTDTKVIGNGSFGVVYQAKLCDSGELVAIKKVLQDKRFKNRELQIMRKLDHCNIVRLRYFFYSSGEKKDEVYLNLVLDYVPETVYRVARHYSRAKQTLPVIYVKLYMYQLFRSLAYIHSFGICHRDIKPQNLLLDPDTAVLKLCDFGSAKQLVRGEPNVSYICSRYYRAPELIFGATDYTSSIDVWSAGCVLAELLLGQPIFPGDSGVDQLVEIIKVLGTPTREQIREMNPNYTEFKFPQIKAHPWTKVFRPRTPPEAIALCSRLLEYTPTARLTPLEACAHSFFDELRDPNVKLPNGRDTPALFNFTTQELSSNPPLATILIPPHARIQAAASTPTNATAASDANTGDRGQTNNAASASASNST

SEQ ID NO: 28 - protein, 433 aa, Homo sapiens
MEVVDPQQLGMFTEGELMSVGMDTFIHRIDSTEVIYQPRRKRAKLIGKYLMGDLLGEGSYGKVKEVLDSETLCRRAVKILKKKKLRRIPNGEANVKKEIQLLRRLRHKNVIQLVDVLYNEEKQKMYMVMEYCVCGMQEMLDSVPEKRFPVCQAHGYFCQLIDGLEYLHSQGIVHKDIKPGNLLLTTGGTLKISDLGVAEALHPFAADDTCRTSQGSPAFQPPEIANGLDTFSGFKVDIWSAGVTLYNITTGLYPFEGDNIYKLFENIGKGSYAIPGDCGPPLSDLLKGMLEYEPAKRFSIRQIRQHSWFRKKHPPAEAPVPIPPSPDTKDRWRSMTVVPYLEDLHGADEDEDLFDIEDDIIYTQDFTVPGQVPEEEASHNGQRRGLPKAVCMNGTEAAQLSTKSRAEGRAPNPARKACSASSKIRRLSACKQQ

SEQ ID NO: 29 - protein, 487 aa, Homo sapiens
METVQLRNPPRRQLKKLDEDSLTKQPEEVFDVLEKLGEGSYGSVYKAIHKETGQIVAIKQVPVESDLQEIIKEISIMQQCDSPHVVKYYGSYFKNTDLWIVMEYCGAGSVSDIIRLRNKTLTEDEIATILQSTLKGLEYLHFMRKIHRDIKAGNILLNTEGHAKLADFGVAGQLTDTMAKRNTVIGTPFWMAPEVIQEIGYNCVADIWSLGITAIEMAEGKPPYADIHPMRAIFMIPTNPPPTFRKPELWSDNFTDFVKQCLVKSPEQRATATQLLQHPFVRSAKGVSILRDLINEAMDVKLKRQESQQREVDQDDEENSEEDEMDSGTMVRAVGDEMGTVRVASTMTDGANTMIEHDDTLPSQLGTMVINAEDEEEEGTMKRRDETMQPAKPSFLEYFEQKEKENQINSFGKSVPGPLKNSSDWKIPQDGDYEFLKSWTVEDLQKRLLALDPMMEQEIEEIRQKYQSKRQPILDAIEAKKRRQQNF

SEQ ID NO: 30 - protein, 445 aa, Homo sapiens
MPSRAEDYEVLYTIGTGSYGRCQKIRRKSDGKILVWKELDYGSMTEAEKQMLVSEVNLLRELKHPNIVRYYDRIIDRTNTTLYIVMEYCEGGDLASVITKGTKERQYLDEEFVLRVMTQLTLALKECHRRSDGGHTVLHRDLKPANVFLDGKQNVKLGDFGLARILNHDTSFAKTFVGTPYYMSPEQMNRMSYNEKSDIWSLGCLLYELCALMPPFTAFSQKELAGKIREGKFRRIPYRYSDELNEIITRMLNLKDYHRPSVEEILENPLIADLVADEQRRNLERRGRQLGEPEKSQDSSPVLSELKLKEIQLQERERALKAREERLEQKEQELCVRERLAEDKLARAENLLKNYSLLKERKFLSLASNPELLNLPSSVIKKKVHFSGESKENIMRSENSESQLTSKSKCKDLKKRLHAAQLRAQALSDIEKNYQLKSRQILGMR

SEQ ID NO: 31 - protein, 591 aa, Homo sapiens
MFGKRKKRVEISAPSNFEHRVHTGFDQHEQKFTGLPRQWQSLIEESARRPKPLVDPACITSIQPGAPKTIVRGSKGAKDGALTLLLDEFENMSVTRSNSLRRDSPPPPARARQENGMPEEPATTARGGPGKAGSRGRFAGHSEAGGGSGDRRRAGPEKRPKSSREGSGGPQESSRDKRPLSGPDVGTPQPAGLASGAKLAAGRPFNTYPRADTDHPSRGAQGEPHDVAPNGPSAGGLAIPQSSSSSSRPPTRARGAPSPGVLGPHASEPQLAPPACTPAAPAVPGPPGPRSPQREPQRVSHEQFRAALQLVVDPGDPRSYLDNFIKIGEGSTGIVCIATVRSSGKLVAVKKMDLRKQQRRELLFNEVVIMRDYQHENVVEMYNSYLVGDELWVVMEFLEGGALTDIVTHTRMNEEQIAAVCLAVLQALSVLHAQGVIHRDIKSDSILLTHDGRVKLSDFGFCAQVSKEVPRRKSLVGTPYWMAPELISRLPYGPEVDIWSLGIMVIEMVDGEPPYFNEPPLKAMKMIRDNLPPRLKNLHKVSPSLKGFLDRLLVRDPAQRATAAELLKHPFLAKAGPPASIVPLMRQNRTR

SEQ ID NO: 32 - protein, 671 aa, Homo sapiens
MADPAAGPPPSEGEESTVRFARKGALRQKNVHEVKNHKFTARFFKQPTFCSHCTDFIWGFGKQGFQCQVCCFVVHKRCHEFVTFSCPGADKGPASDDPRSKHKFKIHTYSSPTFCDHCGSLLYGLIHQGMKCDTCMMNVHKRCVMNVPSLCGTDHTERRGRIYIQAHIDRDVLIVLVRDAKNLVPMDPNGLSDPYVKLKLIPDPKSESKQKTKTIKCSLNPEWNETFRFQLKESDKDRRLSVEIWDWDLTSRNDFMGSLSFGISELQKASVDGWFKLLSQEEGEYFNVPVPPEGSEANEELRQKFERAKISQGTKVPEEKTTNTVSKFDNNGNRDRMKLTDFNFLMVLGKGSFGKVMLSERKGTDELYAVKILKKDVVIQDDDVECTMVEKRVLALPGKPPFLTQLHSCFQTMDRLYFVMEYVNGGDLMYHIQQVGRFKEPHAVFYAAEIAIGLFFLQSKGIIYRDLKLDNVMLDSEGHIKIADFGMCKENIWDGVTTKTFCGTPDYIAPEIIAYQPYGKSVDWWAFGVLLYEMLAGQAPFEGEDEDELFQSIMEHNVAYPKSMSKEAVAICKGLMTKHPGKRLGCGPEGERDIKEHAFFRYIDWEKLERKEIQPPYKPKARDKRDTSNFDKEFTRQPVELTPTDKLFIMNLDQNEFAGFSYTNPEFVINV

SEQ ID NO: 33 - protein, 525 aa, Homo sapiens
MRRRRRRDGFYPAPDFRDREAEDMAGVFDIDLDQPEDAGSEDELEEGGQLNESMDHGGVGPYELGMEHCEKFEISETSVNRGPEKIRPECFELLRVLGKGGYGKVFQVRKVTGANTGKIFAMKVLKKAMIVRNAKDTAHTKAERNILEEVKHPFIVDLIYAFQTGGKLYLILEYLSGGELFMQLEREGIFMEDTACFYLAEISMALGHLHQKGIIYRDLKPENIMLNHQGHVKLTDFGLCKESIHDGTVTHTFCGTIEYMAPEILMRSGHNRAVDWWSLGALMYDMLTGAPPFTGENRKKTIDKILKCKLNLPPYLTQEARDLLKKLLKRNAASRLGAGPGDAGEVQAHPFFRHINWEELLARKVEPPFKPLLQSEEDVSQFDSKFTRQTPVDSPDDSTLSESANQVFLGFTYVAPSVLESVKEKFSFEPKIRSPRRFIGSPRTPVSPVKFSPGDFWGRGASASTANPQTPVEYPMETSGIEQMDVTMSGEASAPLPIRQPNSGPYKKQAFPMISKRPEHLRMNL

SEQ ID NO: 34 - protein, 396 aa, Homo sapiens
MPRVKAAQAGRQSSAKRHLAEQFAVGEIITDMAKKEWKVGLPIGQGGFGCIYLADMNSSESVGSDAPCVVKVEPSDNGPLFTELKFYQRAAKPEQIQKWIRTRKLKYLGVPKYWGSGLHDKNGKSYRFMIMDRFGSDLQKIYEANAKRFSRKTVLQLSLRILDILEYIHEHEYVHGDIKASNLLLNYKNPDQVYLVDYGLAYRYCPEGVHKEYKEDPKRCHDGTIEFTSIDAHNGVAPSRRGDLEILGYCMIQWLTGHLPWEDNLKDPKYVRDSKIRYRENIASLMDKCFPEKNKPGEIAKYMETVKLLDYTEKPLYENLRDILLQGLKAIGSKDDGKLDLSVVENGGLKAKTITKKRKKEIEESKEPGVEDTEWSNTQTEEAIQTRSRTRKRVQK